European Patent Application EP 4 317 208 A1, published February 7, 2024. Title: Aminatoin Method for Polystyrene-type Resin, and Method for Immobilizing Enzyme Using Aminated Resin. Applicant: ASYMCHEM LABORATORIES(TIANJIN)CO.,LTD. The sequence listing filed with the application follows.

SEQUENCE LISTING (1 sequence)

SEQ ID NO: 1 - protein, 459 aa, Chromobacterium violaceum DSM30191
MQKQRTCSQWRELDAAHHLHPFTDTASLNQAGARVMTRGEGVYLWDCEGNKIIDGMAGLWCVNVGYGRKDFAEAARRQMEELPFYNTFFGTTHPPVVELSSLLAEVTPAGFDRVFYTNSGSESVDTMIRMVRRYWDVQGKPEKKTLIGRWNGYHGSTIGGASLGGMKYMHEQGDLPIPGMAHIEQPWWYKHGKDMTPDEFGVVAARWLEEKILEIGADKVAAFVGEPIQGAGGVIVPPATYWPEIERICRKYDVLLVADEVICGFGRTGEWFGHQHFGFQPDLFTAAKGLSSGYLPLGAVFVGDRVAEGLIAGGDFNHGFTYSGHPVCAAVAHANVAALRDEGIVQRVKDDIGPYMQKRWRETFSRFEHVDDVRGVGMMLAFTLVKNKAKRELFPDFGEIGTLCEDIFFRNNLIMTAQGDHIVSAPPLVMTRAEVDEMLAVAERCLEEFEQTLKARGLA